European Patent Application EP 4 772 638 A1, published July 8, 2026. Title: Functional oligonucleotides for enhanced translation of specific proteins through bridging RNAs. Applicant: Kemijski Institut, National Institute of Chemistry, Ljubljana. Application EP. The sequence listing filed with the application follows.

SEQUENCE LISTING (19 sequences)

SEQ ID NO: 1 - RNA, 18 nt, synthetic construct
  source 1..18: mol_type = other RNA
ttcgctctctggcggccc

SEQ ID NO: 2 - RNA, 19 nt, synthetic construct
  source 1..19: mol_type = other RNA
ggttgctgcttcgcgactg

SEQ ID NO: 3 - RNA, 18 nt, synthetic construct
  source 1..18: mol_type = other RNA
ggcccgggcccgcagcgt

SEQ ID NO: 4 - RNA, 18 nt, synthetic construct
  source 1..18: mol_type = other RNA
tttaatggccttgttata

SEQ ID NO: 5 - RNA, 19 nt, synthetic construct
  source 1..19: mol_type = other RNA
ggttgctgcttcgcgactg

SEQ ID NO: 6 - RNA, 19 nt, synthetic construct
  source 1..19: mol_type = other RNA
tcgatgtaagagaacctgc

SEQ ID NO: 7 - RNA, 20 nt, synthetic construct
  source 1..20: mol_type = other RNA
ggcggtcgatgtaagagaac

SEQ ID NO: 8 - RNA, 18 nt, synthetic construct
  source 1..18: mol_type = other RNA
gcgactcttaggcggtcg

SEQ ID NO: 9 - RNA, 18 nt, synthetic construct
  source 1..18: mol_type = other RNA
cttggcaggaagagagtt

SEQ ID NO: 10 - RNA, 19 nt, synthetic construct
  source 1..19: mol_type = other RNA
cggctctggcctacttttc

SEQ ID NO: 11 - RNA, 18 nt, synthetic construct
  source 1..18: mol_type = other RNA
cttctcttcggtccgctg

SEQ ID NO: 12 - RNA, 20 nt, synthetic construct
  source 1..20: mol_type = other RNA
cgaaagatgctacggcgaag

SEQ ID NO: 13 - RNA, 21 nt, synthetic construct
  source 1..21: mol_type = other RNA
ggctgcgttaggcaaggaaag

SEQ ID NO: 14 - RNA, 19 nt, synthetic construct
  source 1..19: mol_type = other RNA
ggcaaggaaagaggacctc

SEQ ID NO: 15 - RNA, 18 nt, synthetic construct
  source 1..18: mol_type = other RNA
cctccgtcttccggtgcg

SEQ ID NO: 16 - RNA, 18 nt, synthetic construct
  source 1..18: mol_type = other RNA
ccggtgcgcgtagaaatt

SEQ ID NO: 17 - RNA, 18 nt, synthetic construct
  source 1..18: mol_type = other RNA
gaccgtcctcgacctgcg

SEQ ID NO: 18 - RNA, 18 nt, synthetic construct
  source 1..18: mol_type = other RNA
tatacttcaaataccctc

SEQ ID NO: 19 - RNA, 18 nt, synthetic construct
  source 1..18: mol_type = other RNA
caggggaacaggctcctc